European Patent Specification EP 3 541 422 B1, published July 1, 2026. Title: METHOD OF TREATING PSORIASIS WITH ANTI-IL23 SPECIFIC ANTIBODY. Applicant: JANSSEN BIOTECH, INC. FITZGERALD, DENNIS JAY SIEGEL YIELDING, NEWMAN. Application Unknown. The sequence listing filed with the application follows.

SEQUENCE LISTING (156 sequences)

SEQ ID NO: 1 - protein, 5 aa, Homo sapiens
NYAIS

SEQ ID NO: 2 - protein, 5 aa, Homo sapiens
SNYIS

SEQ ID NO: 3 - protein, 5 aa, Homo sapiens
NYWIS

SEQ ID NO: 4 - protein, 5 aa, Homo sapiens
SYWIT

SEQ ID NO: 5 - protein, 5 aa, Homo sapiens
NYWIG

SEQ ID NO: 6 - protein, 5 aa, Homo sapiens
SFGMS

SEQ ID NO: 7 - protein, 17 aa, Homo sapiens
GIIPMFGYANYAQKFQG

SEQ ID NO: 8 - protein, 17 aa, Homo sapiens
GIIPVFGFTHYAQKFQG

SEQ ID NO: 9 - protein, 17 aa, Homo sapiens
GIIPIFGHANYAQKFQG

SEQ ID NO: 10 - protein, 17 aa, Homo sapiens
IIIPPIGNAWYAQKFQG

SEQ ID NO: 11 - protein, 17 aa, Homo sapiens
LIDPNFGGAYYAQKFQG

SEQ ID NO: 12 - protein, 17 aa, Homo sapiens
LIDPVFGGAYYAQKFQG

SEQ ID NO: 13 - protein, 17 aa, Homo sapiens
LIDPMFGGAYYAQKFQG

SEQ ID NO: 14 - protein, 16 aa, Homo sapiens
INAHLGGTWYAQKFQG

SEQ ID NO: 15 - protein, 17 aa, Homo sapiens
ISPGTGINAYYAQKFQG

SEQ ID NO: 16 - protein, 17 aa, Artificial Sequence
  Synthesized human sequence
  unsure (1): Where Xaa can be G, I, or L
  unsure (2): Where Xaa can be I or S
  unsure (3): Where Xaa can be I, P, N, or D
  unsure (4): Where Xaa can be P, G, or A
  unsure (5): Where Xaa can be I, M, P,; T, H, N, or V
  unsure (6): Where Xaa can be F, I, G, or L
  unsure (7): Where Xaa can G or I
  unsure (8): Where Xaa can be H, Y, N, or G
  unsure (9): Where Xaa can be A or T
  unsure (10): Where Xaa can be N, W, or Y
XXXXXXXXXXYAQKFQG

SEQ ID NO: 17 - protein, 17 aa, Homo sapiens
WIRPGDSDTRYSPSFEG

SEQ ID NO: 18 - protein, 19 aa, Homo sapiens
VSYISSSGSSTYYADSVKG

SEQ ID NO: 19 - protein, 17 aa, Homo sapiens
IIDPSNSYTNYSPSFQG

SEQ ID NO: 20 - protein, 17 aa, Homo sapiens
IIDPSNSYTRYSPSFQG

SEQ ID NO: 21 - protein, 17 aa, Homo sapiens
IIDPSNSYTDYSPSFQG

SEQ ID NO: 22 - protein, 17 aa, Homo sapiens
IISPTGSVTWYSPSFQG

SEQ ID NO: 23 - protein, 17 aa, Homo sapiens
IISPTGSSTWYSPSFQG

SEQ ID NO: 24 - protein, 17 aa, Homo sapiens
FISPDGSHTWYSPSFQG

SEQ ID NO: 25 - protein, 17 aa, Homo sapiens
IISPSGSTTWYSPSFQG

SEQ ID NO: 26 - protein, 17 aa, Homo sapiens
IISPTGSATWYSPSFQG

SEQ ID NO: 27 - protein, 17 aa, Homo sapiens
IIDPVSSWTKYSPSFQG

SEQ ID NO: 28 - protein, 17 aa, Artificial Sequence
  Synthesized human sequence
  unsure (3): Where Xaa can be D or S
  unsure (5): Where Xaa can be S, V, D, or T
  unsure (6): Where Xaa can be N, S, or G
  unsure (8): Where Xaa can be Y, W, T, H, V, S, or A
  unsure (10): Where Xaa can be N, D, R, K, or W
IIXPXXSXTXYSPSFQG

SEQ ID NO: 29 - protein, 17 aa, Homo sapiens
NISSSGSSTYYADSVKG

SEQ ID NO: 30 - protein, 19 aa, Homo sapiens
NIEHKYLNYATYYAASVKG

SEQ ID NO: 31 - protein, 19 aa, Homo sapiens
NIEHKFMGYTTYYAAGVKG

SEQ ID NO: 32 - protein, 19 aa, Homo sapiens
GIEHKYLSYTTHYAASVKG

SEQ ID NO: 33 - protein, 19 aa, Homo sapiens
SIEHKYTGYTTYYAAPVKG

SEQ ID NO: 34 - protein, 19 aa, Homo sapiens
QIEHKYLSYTTLYAASVKG

SEQ ID NO: 35 - protein, 19 aa, Homo sapiens
SIEHKYLSYTTFYAASVKG

SEQ ID NO: 36 - protein, 19 aa, Homo sapiens
NIEGKYTSYTTYYAASVKG

SEQ ID NO: 37 - protein, 19 aa, Homo sapiens
GIEHKYLSYATLYAASVKG

SEQ ID NO: 38 - protein, 19 aa, Homo sapiens
NIEHKYLGYATVYAASVKG

SEQ ID NO: 39 - protein, 19 aa, Homo sapiens
SIEHKYLSYATYYAAGVKG

SEQ ID NO: 40 - protein, 8 aa, Homo sapiens
DIYAGMDV

SEQ ID NO: 41 - protein, 18 aa, Homo sapiens
SKKGMYGGWTYPLMMFDL

SEQ ID NO: 42 - protein, 7 aa, Homo sapiens
HYYGMDY

SEQ ID NO: 43 - protein, 12 aa, Homo sapiens
GTFWSFGNYFAN

SEQ ID NO: 44 - protein, 8 aa, Homo sapiens
WYYKPFDV

SEQ ID NO: 45 - protein, 12 aa, Homo sapiens
YWGTPYLMQFDN

SEQ ID NO: 46 - protein, 12 aa, Homo sapiens
RASQSVLGNYLA

SEQ ID NO: 47 - protein, 12 aa, Homo sapiens
RASQSVSSNYLA

SEQ ID NO: 48 - protein, 13 aa, Homo sapiens
SGSSSNIGSYYVN

SEQ ID NO: 49 - protein, 11 aa, Homo sapiens
RASQSIFYNLA

SEQ ID NO: 50 - protein, 14 aa, Homo sapiens
TGSSSNIGSGYDVH

SEQ ID NO: 51 - protein, 14 aa, Homo sapiens
TGTSSDVGGYNSVS

SEQ ID NO: 52 - protein, 7 aa, Homo sapiens
GASSRAT

SEQ ID NO: 53 - protein, 7 aa, Homo sapiens
YASRRAT

SEQ ID NO: 54 - protein, 7 aa, Homo sapiens
GNTHRPS

SEQ ID NO: 55 - protein, 7 aa, Homo sapiens
GASNRAT

SEQ ID NO: 56 - protein, 7 aa, Homo sapiens
GNSKRPS

SEQ ID NO: 57 - protein, 7 aa, Homo sapiens
SVSSRPS

SEQ ID NO: 58 - protein, 9 aa, Homo sapiens
HQYGSISTT

SEQ ID NO: 59 - protein, 9 aa, Homo sapiens
QQYSHLLIT

SEQ ID NO: 60 - protein, 9 aa, Homo sapiens
QQYSHISLT

SEQ ID NO: 61 - protein, 9 aa, Homo sapiens
QQFAHILLT

SEQ ID NO: 62 - protein, 9 aa, Homo sapiens
QQTSNTPFT

SEQ ID NO: 63 - protein, 9 aa, Homo sapiens
QQFITYLPT

SEQ ID NO: 64 - protein, 9 aa, Homo sapiens
QQDALSPFT

SEQ ID NO: 65 - protein, 9 aa, Homo sapiens
QQDRGTPFT

SEQ ID NO: 66 - protein, 9 aa, Homo sapiens
QQSLNIPFT

SEQ ID NO: 67 - protein, 9 aa, Homo sapiens
QQDTSSPFT

SEQ ID NO: 68 - protein, 10 aa, Artificial Sequence
  Synthesized human sequence
  unsure (3): Where Xaa can be T, F, D, or S
  unsure (4): Where Xaa can be S, I, A, T, R, or L
  unsure (5): Where Xaa can be N, T, L, S, or G
  unsure (6): Where Xaa can be T, Y, S, or I
  unsure (7): Where Xaa can be P or L
  unsure (8): Where Xaa can be F or P
QQXXXXXXFT

SEQ ID NO: 69 - protein, 11 aa, Homo sapiens
QTYASLGPGEV

SEQ ID NO: 70 - protein, 9 aa, Homo sapiens
QQYSSEPVT

SEQ ID NO: 71 - protein, 9 aa, Homo sapiens
SSWTPSSVV

SEQ ID NO: 72 - protein, 11 aa, Homo sapiens
SSWTDTPNMIV

SEQ ID NO: 73 - protein, 11 aa, Homo sapiens
ASWTDGLSLVV

SEQ ID NO: 74 - protein, 11 aa, Artificial Sequence
  Synthesized human sequence
  unsure (1): Where Xaa can be S or A
  unsure (6): Where Xaa can be T or G
  unsure (7): Where Xaa can be P or L
  unsure (8): Where Xaa can be S or N
  unsure (9): Where Xaa can be S, M, or L
  unsure (10): Where Xaa can be I or V
XSWTDXXXXXV

SEQ ID NO: 75 - protein, 11 aa, Homo sapiens
SSYDTNKPLVV

SEQ ID NO: 76 - protein, 11 aa, Homo sapiens
GSYDVYGRFYV

SEQ ID NO: 77 - protein, 11 aa, Homo sapiens
SSYYFYLQRIV

SEQ ID NO: 78 - protein, 11 aa, Homo sapiens
QTYYFSYSGPV

SEQ ID NO: 79 - protein, 11 aa, Homo sapiens
GSWDPIFSYEV

SEQ ID NO: 80 - protein, 117 aa, Homo sapiens
QVQLVQSGAEVKKPGSSVKVSCKASGGTFSNYAISWVRQAPGQGLEWMGGIIPMFGYANYAQKFQGRVTITADESTSTAYMELSSLRSEDTAVYYCARDIYAGMDVWGQGTLVTVSS

SEQ ID NO: 81 - protein, 117 aa, Homo sapiens
QVQLVQSGAEVKKPGSSVKVSCKASGGTFSNYAISWVRQAPGQGLEWMGGIIPVFGFTHYAQKFQGRVTITADESTSTAYMELSSLRSEDTAVYYCARDIYAGMDVWGQGTLVTVSS

SEQ ID NO: 82 - protein, 108 aa, Homo sapiens
DIVLTQSPATLSLSPGERATLSCRASQSVLGNYLAWYQQKPGQAPRLLIYGASSRATGVPARFSGSGSGTDFTLTISSLEPEDFAVYYCHQYGSISTTFGQGTKVEIK

SEQ ID NO: 83 - protein, 108 aa, Homo sapiens
DIVLTQSPATLSLSPGERATLSCRASQSVLGNYLAWYQQKPGQAPRLLIYGASSRATGVPARFSGSGSGTDFTLTISSLEPEDFAVYYCQQYSHISLTFGQGTKVEIK

SEQ ID NO: 84 - protein, 108 aa, Homo sapiens
DIVLTQSPATLSLSPGERATLSCRASQSVLGNYLAWYQQKPGQAPRLLIYGASSRATGVPARFSGSGSGTDFTLTISSLEPEDFAVYYCQQYSHLIITFGQGTKVEIK

SEQ ID NO: 85 - protein, 108 aa, Homo sapiens
DIVLTQSPATLSLSPGERATLSCRASQSVLGNYLAWYQQKPGQAPRLLIYGASSRATGVPARFSGSGSGTDFTLTISSLEPEDFAVYYCQQFAHILLTFGQGTKVEIK

SEQ ID NO: 86 - protein, 127 aa, Homo sapiens
QVQLVQSGAEVKKPGSSVKVSCKASGGTFSSNYISWVRQAPGQGLEWMGGIIPIFGHANYAQKFQGRVTITADESTSTAYMELSSLRSEDTAVYYCARSKKGMYGGWTYPLMMFDLWGQGTLVTVSS

SEQ ID NO: 87 - protein, 127 aa, Homo sapiens
QVQLVQSGAEVKKPGSSVKVSCKASGGTFSSNYISWVRQAPGQGLEWMGIIIPPIGNAWYAQKFQGRVTITADESTSTAYMELSSLRSEDTAVYYCARSKKGMYGGWTYPLMMFDLWGQGTLVTVSS

SEQ ID NO: 88 - protein, 127 aa, Homo sapiens
QVQLVQSGAEVKKPGSSVKVSCKASGGTFSSNYISWVRQAPGQGLEWMGISPGTGINAYYAQKFQGRVTITADESTSTAYMELSSLRSEDTAVYYCARSKKGMYGGWTYPLMMFDLWGQGTLVTVSS

SEQ ID NO: 89 - protein, 126 aa, Homo sapiens
QVQLVQSGAEVKKPGSSVKVSCKASGGTFSSNYISWVRQAPGQGLEWMGINAHLGGTWYAQKFQGRVTITADESTSTAYMELSSLRSEDTAVYYCARSKKGMYGGWTYPLMMFDLWGQGTLVTVSS

SEQ ID NO: 90 - protein, 127 aa, Homo sapiens
QVQLVQSGAEVKKPGSSVKVSCKASGGTFSSNYISWVRQAPGQGLEWMGLIDPNFGGAYYAQKFQGRVTITADESTSTAYMELSSLRSEDTAVYYCARSKKGMYGGWTYPLMMFDLWGQGTLVTVSS

SEQ ID NO: 91 - protein, 127 aa, Homo sapiens
QVQLVQSGAEVKKPGSSVKVSCKASGGTFSSNYISWVRQAPGQGLEWMGLIDPVFGGAYYAQKFQGRVTITADESTSTAYMELSSLRSEDTAVYYCARSKKGMYGGWTYPLMMFDLWGQGTLVTVSS

SEQ ID NO: 92 - protein, 127 aa, Homo sapiens
QVQLVQSGAEVKKPGSSVKVSCKASGGTFSSNYISWVRQAPGQGLEWMGLIDPMFGGAYYAQKFQGRVTITADESTSTAYMELSSLRSEDTAVYYCARSKKGMYGGWTYPLMMFDLWGQGTLVTVSS

SEQ ID NO: 93 - protein, 108 aa, Homo sapiens
DIVLTQSPATLSLSPGERATLSCRASQSVSSNYLAWYQQKPGQAPRLLIYYASRRATGVPARFSGSGSGTDFTLTISSLEPEDFATYYCQQTSNTPFTFGQGTKVEIK

SEQ ID NO: 94 - protein, 108 aa, Homo sapiens
EIVLTQSPATLSLSPGERATLSCRASQSVSSNYLAWYQQKPGQAPRLLIYYASRRATGVPARFSGSGSGTDFTLTISSLEPEDFAVYYCQQTSNTPFTFGQGTKVEIK

SEQ ID NO: 95 - protein, 108 aa, Homo sapiens
DIVLTQSPATLSLSPGERATLSCRASQSVSSNYLAWYQQKPGQAPRLLIYYASRRATGVPARFSGSGSGTDFTLTISSLEPEDFAVYYCQQFITYLPTFGQGTKVEIK

SEQ ID NO: 96 - protein, 108 aa, Homo sapiens
DIVLTQSPATLSLSPGERATLSCRASQSVSSNYLAWYQQKPGQAPRLLIYYASRRATGVPARFSGSGSGTDFTLTISSLEPEDFAVYYCQQDALSPFTFGQGTKVEIK

SEQ ID NO: 97 - protein, 108 aa, Homo sapiens
DIVLTQSPATLSLSPGERATLSCRASQSVSSNYLAWYQQKPGQAPRLLIYYASRRATGVPARFSGSGSGTDFTLTISSLEPEDFAVYYCQQDRGTPFTFGQGTKVEIK

SEQ ID NO: 98 - protein, 108 aa, Homo sapiens
DIVLTQSPATLSLSPGERATLSCRASQSVSSNYLAWYQQKPGQAPRLLIYYASRRATGVPARFSGSGSGTDFTLTISSLEPEDFAVYYCQQSLNIPFTFGQGTKVEIK

SEQ ID NO: 99 - protein, 116 aa, Homo sapiens
QVQLVQSGAEVKKPGESLKISCKGSGYSFTNYWISWVRQAPGKGLEWMGWIRPGDSDTRYSPSFEGQVTISADKSISTAYLQWSSLKASDTAMYYCARHYYGMDYWGQGTLVTVSS

SEQ ID NO: 100 - protein, 110 aa, Homo sapiens
DIVLTQPPSVSGAPGQRVTISCSGSSSNIGSYYVNWYQQLPGTAPKLLIYGNTHRPSGVPDRFSGSKSGTSASLAITGLQSEDEADYYCQTYASLGPGEVFGGGTKLTVL

SEQ ID NO: 101 - protein, 121 aa, Homo sapiens
QVQLVESGGGLVQPGGSLRLSCAASGFTFSSYWITWVRQAPGKGLEWVSYISSSGSSTYYADSVKGRFTISRDNSKNTLYLQMNSLRAEDTAVYYCARGTFWSFGNYFANWGQGTLVTVSS

SEQ ID NO: 102 - protein, 107 aa, Homo sapiens
DIVLTQSPATLSLSPGERATLSCRASQSIFYNLAWYQQKPGQAPRLLIYGASNRATGVPARFSGSGSGTDFTLTISSLEPEDFATYYCQQYSSEPVTFGQGTKVEIK

SEQ ID NO: 103 - protein, 117 aa, Homo sapiens
QVQLVQSGAEVKKPGESLKISCKGSGYSFSNYWIGWVRQMPGKGLEWMGIIDPSNSYTNYSPSFQGQVTISADKSISTAYLQWSSLKASDTAMYYCARWYYKPFDVWGQGTLVTVSS

SEQ ID NO: 104 - protein, 117 aa, Homo sapiens
QVQLVQSGAEVKKPGESLKISCKGSGYSFSNYWIGWVRQMPGKGLEWMGIIDPSNSYTDYSPSFQGQVTISADKSISTAYLQWSSLKASDTAMYYCARWYYKPFDVWGQGTLVTVSS

SEQ ID NO: 105 - protein, 117 aa, Homo sapiens
QVQLVQSGAEVKKPGESLKISCKGSGYSFSNYWIGWVRQMPGKGLEWMGIIDPSNSYTRYSPSFQGQVTISADKSISTAYLQWSSLKASDTAMYYCARWYYKPFDVWGQGTLVTVSS

SEQ ID NO: 106 - protein, 117 aa, Homo sapiens
EVQLVQSGAEVKKPGESLKISCKGSGYSFSNYWIGWVRQMPGKGLEWMGIIDPSNSYTRYSPSFQGQVTISADKSISTAYLQWSSLKASDTAMYYCARWYYKPFDVWGQGTLVTVSS

SEQ ID NO: 107 - protein, 117 aa, Homo sapiens
QVQLVQSGAEVKKPGESLKISCKGSGYSFSNYWIGWVRQMPGKGLEWMGIIDPVSSWTKYSPSFQGQVTISADKSISTAYLQWSSLKASDTAMYYCARWYYKPFDVWGQGTLVTVSS

SEQ ID NO: 108 - protein, 117 aa, Homo sapiens
QVQLVQSGAEVKKPGESLKISCKGSGYSFSNYWIGWVRQMPGKGLEWMGIISPSGSTTWYSPSFQGQVTISADKSISTAYLQWSSLKASDTAMYYCARWYYKPFDVWGQGTLVTVSS

SEQ ID NO: 109 - protein, 117 aa, Homo sapiens
QVQLVQSGAEVKKPGESLKISCKGSGYSFSNYWIGWVRQMPGKGLEWMGFISPDGSHTWYSPSFQGQVTISADKSISTAYLQWSSLKASDTAMYYCARWYYKPFDVWGQGTLVTVSS

SEQ ID NO: 110 - protein, 117 aa, Homo sapiens
QVQLVQSGAEVKKPGESLKISCKGSGYSFSNYWIGWVRQMPGKGLEWMGIISPTGSVTWYSPSFQGQVTISADKSISTAYLQWSSLKASDTAMYYCARWYYKPFDVWGQGTLVTVSS

SEQ ID NO: 111 - protein, 117 aa, Homo sapiens
QVQLVQSGAEVKKPGESLKISCKGSGYSFSNYWIGWVRQMPGKGLEWMGIISPTGSSTWYSPSFQGQVTISADKSISTAYLQWSSLKASDTAMYYCARWYYKPFDVWGQGTLVTVSS

SEQ ID NO: 112 - protein, 117 aa, Homo sapiens
QVQLVQSGAEVKKPGESLKISCKGSGYSFSNYWIGWVRQMPGKGLEWMGIISPTGSATWYSPSFQGQVTISADKSISTAYLQWSSLKASDTAMYYCARWYYKPFDVWGQGTLVTVSS

SEQ ID NO: 113 - protein, 109 aa, Homo sapiens
DIVLTQPPSVSGAPGQRVTISCTGSSSNIGSGYDVHWYQQLPGTAPKLLIYGNSKRPSGVPDRFSGSKSGTSASLAITGLQSEDEADYYCSSWTPSSVVFGGGTKLTVL

SEQ ID NO: 114 - protein, 111 aa, Homo sapiens
DIVLTQPPSVSGAPGQRVTISCTGSSSNIGSGYDVHWYQQLPGTAPKLLIYGNSKRPSGVPDRFSGSKSGTSASLAITGLQSEDEADYYCSSWTDTPNMIVFGGGTKLTVL

SEQ ID NO: 115 - protein, 111 aa, Homo sapiens
DIVLTQPPSVSGAPGQRVTISCTGSSSNIGSGYDVHWYQQLPGTAPKLLIYGNSKRPSGVPDRFSGSKSGTSASLAITGLQSEDEADYYCASWTDGLSLVVFGGGTKLTVL

SEQ ID NO: 116 - protein, 111 aa, Homo sapiens
QSVLTQPPSVSGAPGQRVTISCTGSSSNIGSGYDVHWYQQLPGTAPKLLIYGNSKRPSGVPDRFSGSKSGTSASLAITGLQSEDEADYYCASWTDGLSLVVFGGGTKLTVL

SEQ ID NO: 117 - protein, 121 aa, Homo sapiens
QVQLVESGGGLVQPGGSLRLSCAASGFTFSSFGMSWVRQAPGKGLEWVSNISSSGSSTYYADSVKGRFTISRDNSKNTLYLQMNSLRAEDTAVYYCARYWGTPYLMQFDNWGQGTLVTVSS

SEQ ID NO: 118 - protein, 123 aa, Homo sapiens
QVQLVESGGGLVQPGGSLRLSCAASGFTFSSFGMSWVRQAPGKGLEWVSNIEHKFMGYTTYYAAGVKGRFTISRDNSKNTLYLQMNSLRAEDTAVYYCARYWGTPYLMQFDNWGQGTLVTVSS

SEQ ID NO: 119 - protein, 123 aa, Homo sapiens
QVQLVESGGGLVQPGGSLRLSCAASGFTFSSFGMSWVRQAPGKGLEWVSSIEHKYTGYTTYYAAPVKGRFTISRDNSKNTLYLQMNSLRAEDTAVYYCARYWGTPYLMQFDNWGQGTLVTVSS

SEQ ID NO: 120 - protein, 123 aa, Homo sapiens
QVQLVESGGGLVQPGGSLRLSCAASGFTFSSFGMSWVRQAPGKGLEWVSNIEHKYTSYTTYYAASVKGRFTISRDNSKNTLYLQMNSLRAEDTAVYYCARYWGTPYLMQFDNWGQGTLVTVSS

SEQ ID NO: 121 - protein, 123 aa, Homo sapiens
QVQLVESGGGLVQPGGSLRLSCAASGFTFSSFGMSWVRQAPGKGLEWVSNIEHKYLNYATYYAASVKGRFTISRDNSKNTLYLQMNSLRAEDTAVYYCARYWGTPYLMQFDNWGQGTLVTVSS

SEQ ID NO: 122 - protein, 123 aa, Homo sapiens
QVQLVESGGGLVQPGGSLRLSCAASGFTFSSFGMSWVRQAPGKGLEWVSNIEHKYLGYATVYAASVKGRFTISRDNSKNTLYLQMNSLRAEDTAVYYCARYWGTPYLMQFDNWGQGTLVTVSS

SEQ ID NO: 123 - protein, 123 aa, Homo sapiens
QVQLVESGGGLVQPGGSLRLSCAASGFTFSSFGMSWVRQAPGKGLEWVSSIEHKYLSYATYYAAGVKGRFTISRDNSKNTLYLQMNSLRAEDTAVYYCARYWGTPYLMQFDNWGQGTLVTVSS

SEQ ID NO: 124 - protein, 123 aa, Homo sapiens
QVQLVESGGGLVQPGGSLRLSCAASGFTFSSFGMSWVRQAPGKGLEWVSSIEHKYLSYTTFYAASVKGRFTISRDNSKNTLYLQMNSLRAEDTAVYYCARYWGTPYLMQFDNWGQGTLVTVSS

SEQ ID NO: 125 - protein, 123 aa, Homo sapiens
QVQLVESGGGLVQPGGSLRLSCAASGFTFSSFGMSWVRQAPGKGLEWVSGIEHKYLSYTTHYAASVKGRFTISRDNSKNTLYLQMNSLRAEDTAVYYCARYWGTPYLMQFDNWGQGTLVTVSS

SEQ ID NO: 126 - protein, 123 aa, Homo sapiens
QVQLVESGGGLVQPGGSLRLSCAASGFTFSSFGMSWVRQAPGKGLEWVSQIEHKYLSYTTLYAASVKGRFTISRDNSKNTLYLQMNSLRAEDTAVYYCARYWGTPYLMQFDNWGQGTLVTVSS

SEQ ID NO: 127 - protein, 123 aa, Homo sapiens
QVQLVESGGGLVQPGGSLRLSCAASGFTFSSFGMSWVRQAPGKGLEWVSGIEHKYLSYATLYAASVKGRFTISRDNSKNTLYLQMNSLRAEDTAVYYCARYWGTPYLMQFDNWGQGTLVTVSS

SEQ ID NO: 128 - protein, 111 aa, Homo sapiens
DIALTQPASVSGSPGQSITISCTGTSSDVGGYNSVSWYQQHPGKAPKLMIYSVSSRPSGVSNRFSGSKSGNTASLTISGLQAEDEADYYCSSYDTNKPLVVFGGGTKLTVL

SEQ ID NO: 129 - protein, 111 aa, Homo sapiens
DIALTQPASVSGSPGQSITISCTGTSSDVGGYNSVSWYQQHPGKAPKLMIYSVSSRPSGVSNRFSGSKSGNTASLTISGLQAEDEADYYCSSYYFYLQRIVFGGGTKLTVL

SEQ ID NO: 130 - protein, 111 aa, Homo sapiens
DIALTQPASVSGSPGQSITISCTGTSSDVGGYNSVSWYQQHPGKAPKLMIYSVSSRPSGVSNRFSGSKSGNTASLTISGLQAEDEADYYCQTYYFSYSGPVFGGGTKLTVL

SEQ ID NO: 131 - protein, 111 aa, Homo sapiens
DIALTQPASVSGSPGQSITISCTGTSSDVGGYNSVSWYQQHPGKAPKLMIYSVSSRPSGVSNRFSGSKSGNTASLTISGLQAEDEADYYCGSYDVYGRFYVFGGGTKLTVL

SEQ ID NO: 132 - protein, 111 aa, Homo sapiens
DIALTQPASVSGSPGQSITISCTGTSSDVGGYNSVSWYQQHPGKAPKLMIYSVSSRPSGVSNRFSGSKSGNTASLTISGLQAEDEADYYCGSWDPIFSYEVFGGGTKLTVL

SEQ ID NO: 133 - DNA, 381 bp, Homo sapiens
caggtgcagctggtgcagtctggggctgaggtgaagaagcctgggtcctcggtgaaggtctcctgcaaggcttctggaggcaccttcagcagcaactacatcagctgggtgcgacaggcccctggacaagggcttgagtggatggggatcagccctggcaccggtatcaacgcatactacgcacagaagttccagggcagagtcacgattaccgcggacgaatccacgagcacagcctacatggagctgagcagcctgagatctgaggacacggccgtgtattactgtgcgagaagcaagaagggcatgtacggcggctggacctaccccctgatgatgttcgacctgtggggccagggcaccctggtgaccgtgagcagc

SEQ ID NO: 134 - DNA, 381 bp, Homo sapiens
caggtgcagctggtgcagagcggcgccgaggtgaagaagcccggcagcagcgtgaaggtgagctgcaaggccagcggcggcaccttcagcagcaactacatcagctgggtgcgccaggcccccggccagggcctggagtggatgggcatcagccccggcaccggcatcaacgcctactacgcccagaagttccagggccgcgtgaccatcaccgccgacgagagcaccagcaccgcctacatggagctgagcagcctgcgcagcgaggacaccgccgtgtactactgcgcccgcagcaagaagggcatgtacggcggctggacctaccccctgatgatgttcgacctgtggggccagggcaccctggtgaccgtgagcagc

SEQ ID NO: 135 - DNA, 381 bp, Homo sapiens
caggtgcaattggttcagtctggcgcggaagtgaaaaaaccgggcagcagcgtgaaagtgagctgcaaagcctccggaggcactttttcttctaattatatttcttgggtgcgccaagcccctgggcagggtctcgagtggatgggcatttctcctggtactggtattaatgcttattatgctcagaagtttcagggtcgggtgaccattaccgcggatgaaagcaccagcaccgcgtatatggaactgagcagcctgcgtagcgaagatacggccgtgtattattgcgcgcgttctaagaagggtatgtatggtggttggacttatcctcttatgatgtttgatctttggggccaaggcaccctggtgacggttagctca

SEQ ID NO: 136 - DNA, 324 bp, Homo sapiens
gagatcgtgctgacccagagccccgccaccctgagcctgagccccggcgagcgcgccaccctgagctgccgcgccagccagagcgtgagcagcaactacctggcctggtaccagcagaagcccggccaggccccccgcctgctgatctactacgccagccgccgcgccaccggcgtgcccgcccgcttcagcggcagcggcagcggcaccgacttcaccctgaccatcagcagcctggagcccgaggacttcgccgtgtactactgccagcagaccagcaacacccccttcaccttcggccagggcaccaaggtggagatcaag

SEQ ID NO: 137 - DNA, 324 bp, Homo sapiens
gaaattgtgttgacacagtctccagccaccctgtctttgtctccaggggaaagagccaccctctcctgcagggccagtcagagtgttagcagcaactacttagcctggtaccaacagaaacctggccaggctcccaggctcctcatctattacgcatcccgcagggccactggcgtgccagccaggttcagtggcagtgggtctgggacagacttcactctcaccatcagcagcctagagcctgaagattttgcagtttattactgtcagcagacttctaatactccttttacctttggccagggtacgaaagttgaaattaaa

SEQ ID NO: 138 - DNA, 324 bp, Homo sapiens
gagatcgtgctgacccagagcccggcgaccctgagcctgtctccgggcgaacgtgcgaccctgagctgcagagcgagccagtctgtttcttctaattatctggcttggtaccagcagaaaccaggtcaagcaccgcgtctattaatttattatgcttctcgtcgtgcaactggggtcccggcgcgttttagcggctctggatccggcacggattttaccctgaccattagcagcctggaacctgaagactttgcggtgtattattgccagcagacttctaatactccttttacctttggccagggtacgaaagttgaaattaaa

SEQ ID NO: 139 - DNA, 351 bp, Homo sapiens
gaggtgcagctggtgcagtctggagcagaggtgaaaaagcccggggagtctctgaagatctcctgtaagggttctggatacagctttagcaactactggatcggctgggtgcgccagatgcccgggaaaggcctggagtggatggggatcatcgaccctagcaactcttacaccagatacagcccgtccttccaaggccaggtcaccatctcagccgacaagtccatcagcaccgcctacctgcagtggagcagcctgaaggcctcggacaccgccatgtattactgtgcgagatggtactacaagcccttcgacgtgtggggccagggcaccctggtgaccgtgagcagc

SEQ ID NO: 140 - DNA, 351 bp, Homo sapiens
gaggtgcagctggtgcagagcggcgccgaggtgaagaagcccggcgagagcctgaagatcagctgcaagggcagcggctacagcttcagcaactactggatcggctgggtgcgccagatgcccggcaagggcctggagtggatgggcatcatcgaccccagcaacagctacacccgctacagccccagcttccagggccaggtgaccatcagcgccgacaagagcatcagcaccgcctacctgcagtggagcagcctgaaggccagcgacaccgccatgtactactgcgcccgctggtactacaagcccttcgacgtgtggggccagggcaccctggtgaccgtgagcagc

SEQ ID NO: 141 - DNA, 351 bp, Homo sapiens
gaggtgcaattggttcagagcggcgcggaagtgaaaaaaccgggcgaaagcctgaaaattagctgcaaaggttccggatattccttttctaattattggattggttgggtgcgccagatgcctgggaagggtctcgagtggatgggcattatcgatccgtctaatagctatacccgctattctccgagctttcagggccaggtgaccattagcgcggataaaagcattagcaccgcgtatcttcaatggagcagcctgaaagcgagcgatacggccatgtattattgcgcgcgttggtattataagccttttgatgtttggggccaaggcaccctggtgacggttagctca

SEQ ID NO: 142 - DNA, 336 bp, Homo sapiens
cagtctgtgctgacgcagccgccctcagtgtctggggccccagggcagagggtcaccatctcctgcactgggagcagctccaacatcgggagcggttatgatgtacactggtaccagcagcttccaggaacagcccccaaactcctcatctatggtaacagcaagcggccctcaggggtccctgaccgattctctggctccaagtctggcacctcagcctccctggccatcactgggctccagagcgaggatgaggctgattattactgcgccagctggaccgacggcctgagcctggtggtgttcggcggcggcaccaagctgaccgtgctgggc

SEQ ID NO: 143 - DNA, 336 bp, Homo sapiens
cagagcgtgctgacccagccccccagcgtgagcggcgcccccggccagcgcgtgaccatcagctgcaccggcagcagcagcaacatcggcagcggctacgacgtgcactggtaccagcagctgcccggcaccgcccccaagctgctgatctacggcaacagcaagcgccccagcggcgtgcccgaccgcttcagcggcagcaagagcggcaccagcgccagcctggccatcaccggcctccagagcgaggacgaggccgactactactgtgccagctggaccgacggcctgagcctggtggtgttcggcggcggcaccaagctgaccgtgctgggc

SEQ ID NO: 144 - DNA, 336 bp, Homo sapiens
cagagcgtgctgacccagccgccttcagtgagtggcgcaccaggtcagcgtgtgaccatctcgtgtacgggcagcagcagcaacattggttctggttatgatgtgcattggtaccagcagttgcccgggacggcgccgaaacttctgatttatggtaattctaagcgtccctcaggcgtgccggatcgttttagcggatccaaaagcggcaccagcgcgagccttgcgattacgggcctgcaaagcgaagacgaagcggattattattgcgcttcttggactgatggtctttctcttgttgtgtttggcggcggcacgaagttaaccgttcttggc

SEQ ID NO: 145 - protein, 189 aa, Homo sapiens [sequence omitted]

SEQ ID NO: 146 - protein, 19 aa, Homo sapiens
NIEHKYLGYATSYAASVKG

SEQ ID NO: 147 - protein, 123 aa, Homo sapiens
QVQLVESGGGLVQPGGSLRLSCAASGFTFSSFGMSWVRQAPGKGLEWVSNIEHKYLGYATSYAASVKGRFTISRDNSKNTLYLQMNSLRAEDTAVYYCARYWGTPYLMQFDNWGQGTLVTVSS

SEQ ID NO: 148 - protein, 12 aa, Homo sapiens
HQGLIFYEKLLG

SEQ ID NO: 149 - protein, 5 aa, Homo sapiens
TYWLG

SEQ ID NO: 150 - protein, 17 aa, Homo sapiens
IMSPVDSDIRYSPSFQG

SEQ ID NO: 151 - protein, 10 aa, Homo sapiens
RRPGQGYFDF

SEQ ID NO: 152 - protein, 11 aa, Homo sapiens
RASQGISSWLA

SEQ ID NO: 153 - protein, 7 aa, Homo sapiens
AASSLQS

SEQ ID NO: 154 - protein, 9 aa, Homo sapiens
QQYNIYPYT

SEQ ID NO: 155 - protein, 119 aa, Homo sapiens
EVQLVQSGAEVKKPGESLKISCKGSGYSFTTYWLGWVRQMPGKGLDWIGIMSPVDSDIRYSPSFQGQVTMSVDKSITTAYLQWNSLKASDTAMYYCARRRPGQGYFDFWGQGTLVTVSS

SEQ ID NO: 156 - protein, 108 aa, Homo sapiens
DIQMTQSPSSLSASVGDRVTITCRASQGISSWLAWYQQKPEKAPKSLIYAASSLQSGVPSRFSGSGSGTDFTLTISSLQPEDFATYYCQQYNIYPYTFGQGTKLEIKR